European Patent Application EP 4 311 834 A1, published January 31, 2024. Title: Peptides and combinations of peptides for use in immunotherapy against oropharyngeal squamous cell carcinoma (OPSCC) and other cancers. Applicant: Eberhard Karls Universität Tübingen - Medizinische Fakultät. The sequence listing filed with the application follows.

SEQUENCE LISTING (62 sequences)

SEQ ID NO: 1 - protein, 15 aa, synthetic construct
IRQFTSSSSIKGSSG

SEQ ID NO: 2 - protein, 16 aa, synthetic construct
LTSTSGPGFHLMLPFI

SEQ ID NO: 3 - protein, 24 aa, synthetic construct
ELKKKLKEKAKERREKEMLERLEK

SEQ ID NO: 4 - protein, 15 aa, synthetic construct
ENDVIISINGQSVVS

SEQ ID NO: 5 - protein, 15 aa, synthetic construct
IQDFIEAEDDLSSFR

SEQ ID NO: 6 - protein, 16 aa, synthetic construct
PVHWQFGQLDQHPIDG

SEQ ID NO: 7 - protein, 13 aa, synthetic construct
FADFTFATGKIIG

SEQ ID NO: 8 - protein, 25 aa, synthetic construct
IKNIISEYKSAIQSQKRRRPRYRKR

SEQ ID NO: 9 - protein, 15 aa, synthetic construct
VDEEEVKFPGTNFDE

SEQ ID NO: 10 - protein, 17 aa, synthetic construct
TLCEKLTVSLSDPDPVF

SEQ ID NO: 11 - protein, 17 aa, synthetic construct
ARLPIIDLAPVDVGGTD

SEQ ID NO: 12 - protein, 15 aa, synthetic construct
LPIIDLAPVDVGGTD

SEQ ID NO: 13 - protein, 11 aa, synthetic construct
HRGLRHFWGLR

SEQ ID NO: 14 - protein, 16 aa, synthetic construct
LQNKILTATVDNANIL

SEQ ID NO: 15 - protein, 9 aa, synthetic construct
GVLENIFGV

SEQ ID NO: 16 - protein, 9 aa, synthetic construct
KLAEISLGV

SEQ ID NO: 17 - protein, 9 aa, synthetic construct
RLDDLKMTV

SEQ ID NO: 18 - protein, 11 aa, synthetic construct
GLWEDGRSTLL

SEQ ID NO: 19 - protein, 9 aa, synthetic construct
ALLGSAFQL

SEQ ID NO: 20 - protein, 10 aa, synthetic construct
RLLEGEDAHL

SEQ ID NO: 21 - protein, 9 aa, synthetic construct
ALTDIVSQV

SEQ ID NO: 22 - protein, 9 aa, synthetic construct
RLLDSVSRL

SEQ ID NO: 23 - protein, 9 aa, synthetic construct
VLFPNLKTV

SEQ ID NO: 24 - protein, 9 aa, synthetic construct
YLEEFITNI

SEQ ID NO: 25 - protein, 9 aa, synthetic construct
RTEFNLNQY

SEQ ID NO: 26 - protein, 9 aa, synthetic construct
EMEAQNQEY

SEQ ID NO: 27 - protein, 9 aa, synthetic construct
RTDIARTEY

SEQ ID NO: 28 - protein, 11 aa, synthetic construct
YSELASHVVSY

SEQ ID NO: 29 - protein, 9 aa, synthetic construct
EMEQQNQEY

SEQ ID NO: 30 - protein, 9 aa, synthetic construct
VLDSHIHAY

SEQ ID NO: 31 - protein, 9 aa, synthetic construct
GTEDELDKY

SEQ ID NO: 32 - protein, 12 aa, synthetic construct
RLRGGSPLNTGK

SEQ ID NO: 33 - protein, 9 aa, synthetic construct
KYMYFTVVM

SEQ ID NO: 34 - protein, 9 aa, synthetic construct
NWPSRPYLF

SEQ ID NO: 35 - protein, 9 aa, synthetic construct
GYIDNVTLI

SEQ ID NO: 36 - protein, 9 aa, synthetic construct
AVGPPTTVR

SEQ ID NO: 37 - protein, 10 aa, synthetic construct
APAAWLRSAA

SEQ ID NO: 38 - protein, 9 aa, synthetic construct
APKAPGSPW

SEQ ID NO: 39 - protein, 9 aa, synthetic construct
DATETTITI

SEQ ID NO: 40 - protein, 8 aa, synthetic construct
DQYKFLAV

SEQ ID NO: 41 - protein, 9 aa, synthetic construct
VALPVYLLI

SEQ ID NO: 42 - protein, 8 aa, synthetic construct
HGTIKNQL

SEQ ID NO: 43 - protein, 8 aa, synthetic construct
VAAPRWVL

SEQ ID NO: 44 - protein, 9 aa, synthetic construct
EIKFKVETL

SEQ ID NO: 45 - protein, 10 aa, synthetic construct
SASPKEKYSL

SEQ ID NO: 46 - protein, 10 aa, synthetic construct
EETNPKGSGW

SEQ ID NO: 47 - protein, 9 aa, synthetic construct
IEDDPKMMW

SEQ ID NO: 48 - protein, 9 aa, synthetic construct
SEAESRIFW

SEQ ID NO: 49 - protein, 10 aa, synthetic construct
REVVDPEVFF

SEQ ID NO: 50 - protein, 10 aa, synthetic construct
SEPNDVFFKL

SEQ ID NO: 51 - protein, 9 aa, synthetic construct
SEVVDVAKL

SEQ ID NO: 52 - protein, 11 aa, synthetic construct
VEDSALLMQTL

SEQ ID NO: 53 - protein, 11 aa, synthetic construct
MEAPAQLLFLL

SEQ ID NO: 54 - protein, 9 aa, synthetic construct
YTFRYPLSL

SEQ ID NO: 55 - protein, 9 aa, synthetic construct
ARLAFVIVF

SEQ ID NO: 56 - protein, 8 aa, synthetic construct
RQLVFNEI

SEQ ID NO: 57 - protein, 9 aa, synthetic construct
SPEDGIHEL

SEQ ID NO: 58 - protein, 10 aa, synthetic construct
VFDLVELEVL

SEQ ID NO: 59 - protein, 9 aa, synthetic construct
YEIDDVERL

SEQ ID NO: 60 - protein, 9 aa, synthetic construct
SAVKEGTAM

SEQ ID NO: 61 - protein, 9 aa, synthetic construct
YEEAMKEVL

SEQ ID NO: 62 - protein, 9 aa, synthetic construct
ARLIPIIVL